European Patent Application EP 4 144 365 A1, published March 8, 2023. Title: METHOD FOR IMPROVING IMMUNOGENICITY OF PROTEIN/PEPTIDE ANTIGEN. Applicant: SinoCellTech Ltd. The sequence listing filed with the application follows.

SEQUENCE LISTING (19 sequences)

SEQ ID NO: 1 - protein, 223 aa, Artificial
  The sequence is artifically synthesized.
RVQPTESIVRFPNITNLCPFGEVFNATRFASVYAWNRKRISNCVADYSVLYNSASFSTFKCYGVSPTKLNDLCFTNVYADSFVIRGDEVRQIAPGQTGKIADYNYKLPDDFTGCVIAWNSNNLDSKVGGNYNYLYRLFRKSNLKPFERDISTEIYQAGSTPCNGVEGFNCYFPLQSYGFQPTNGVGYQPYRVVVLSFELLHAPATVCGPKKSTNLVKNKCVNF

SEQ ID NO: 2 - protein, 234 aa, Artificial
  The sequence is artificially synthesized.
RVQPTESIVRFPNITNLCPFGEVFNATRFASVYAWNRKRISNCVADYSVLYNSASFSTFKCYGVSPTKLNDLCFTNVYADSFVIRGDEVRQIAPGQTGKIADYNYKLPDDFTGCVIAWNSNNLDSKVGGNYNYLYRLFRKSNLKPFERDISTEIYQAGSTPCNGVEGFNCYFPLQSYGFQPTNGVGYQPYRVVVLSFELLHAPATVCGPKKSTNLVKNKCVNFAHHHHHHHHHH

SEQ ID NO: 3 - protein, 457 aa, Artificial
  The sequence is artificially synthesized.
RVQPTESIVRFPNITNLCPFGEVFNATRFASVYAWNRKRISNCVADYSVLYNSASFSTFKCYGVSPTKLNDLCFTNVYADSFVIRGDEVRQIAPGQTGKIADYNYKLPDDFTGCVIAWNSNNLDSKVGGNYNYLYRLFRKSNLKPFERDISTEIYQAGSTPCNGVEGFNCYFPLQSYGFQPTNGVGYQPYRVVVLSFELLHAPATVCGPKKSTNLVKNKCVNFADDDDKAVPRDSGCKPCICTVPEVSSVFIFPPKPKDVLTITLTPKVTCVVVDISKDDPEVQFSWFVDDVEVHTAQTQPREEQFNSTFRSVSELPIMHQDWLNGKEFKCRVNSAAFPAPIEKTISKTKGRPKAPQVYTIPPPKEQMAKDKVSLTCMITDFFPEDITVEWQWNGQPAENYKNTQPIMDTDGSYFVYSKLNVQKSNWEAGNTFTCSVLHEGLHNHHTEKSLSHSPGK

SEQ ID NO: 4 - protein, 232 aa, Artificial
  The sequence is artificially synthesized.
NHKVTSTTTIIQDATSQIKNTTPTYLTQSPQLGISPSNPSEITSQITTILASTTPGVKSTLQSTTVGTKNTTTTQAQPSKPTTKQRQNKPPSKPNNDFHFEVFNFVPCSICSNNPTCWAICKRIPNKKPGKKTTTKPTEEPTFKTAKEDPKPQTTGSGEVPTTKPTGEPTINTTKTNITTTLLTSNTTRNPELTSQMETFHSTSSEGNPSPSQVSITSEYLSQPSSPPNTPR

SEQ ID NO: 5 - protein, 158 aa, Artificial
  The sequence is artificially synthesized.
ALEVLFQGPYEVRNVSGIYHVTNDCSNSSIVYEAADVIMHTPGCVPCVREGNSSRCWVALTPTLAARNASVPTTTIRRHVDLLVGTAAFCSAMYVGDLCGSIFLVSQLFTFSPRRHETVQDCNCSIYPGHVSGHRMAWDMMMNWSPTTALVVSQLLRI

SEQ ID NO: 6 - protein, 278 aa, Artificial
  The sequence is artificially synthesized.
ETHTTGRVAGHTTSGFTSLFSSGASQKIQLVNTNGSWHINRTALNCNDSLQTGFFAALFYAHKFNSSGCPERMASCRPIDWFAQGWGPITYTKPNSSDQRPYCWHYAPRPCGVVPASQVCGPVYCFTPSPVVVGTTDRSGVPTYSWGENETDMMLLNNTRPPQGNWFGCTWMNSTGFTKTCGGPPCNIGGVGNRTLICPTDCFRKHPEATYTKCGSGPWLTPRCLVDYPYRLWHYPCTLNFSIFKVRMYVGGVEHRLNAACNWTRGERCNLEDRDRSE

SEQ ID NO: 7 - protein, 347 aa, Artificial
  The sequence is artificially synthesized.
DRICTGITSSNSPHVVKTATQGEVNVTGVIPLTTTPTKSHFANLKGTETRGKLCPKCLNCTDLDVALGRPKCTGKIPSARVSILHEVRPVTSGCFPIMHDRTKIRQLPNLLRGYEHIRLSTHNVINAENAPGGPYKIGTSGSCPNITNGNGFFATMAWAVPKNDKNKTATNPLTIEVPYICTEGEDQITVWGFHSDNETQMAKLYGDSKPQKFTSSANGVTTHYVSQIGGFPNQTEDGGLPQSGRIVVDYMVQKSGKTGTITYQRGILLPQKVWCASGRSKVIKGSLPLIGEADCLHEKYGGLNKSKPYYTGEHAKAIGNCPIWVKTPLKLANGTKYRPPAKLLKER

SEQ ID NO: 8 - protein, 511 aa, Artificial
  The sequence is artificially synthesized.
DQICIGYHANNSTEQVDTIMEKNVTVTHAQDILEKTHNGKLCDLDGVKPLILRDCSVAGWLLGNPMCDEFINVPEWSYIVEKANPANDLCYPGNFNDYEELKHLLSRINHFEKIQIIPKSSWSDHEASSGVSSACPYQGTPSFFRNVVWLIKKNNTYPTIKRSYNNTNQEDLLILWGIHHSNDAAEQTKLYQNPTTYISVGTSTLNQRLVPKIATRSKVNGQSGRMDFFWTILKPNDAINFESNGNFIAPEYAYKIVKKGDSAIVKSEVEYGNCNTKCQTPIGAINSSMPFHNIHPLTIGECPKYVKSNKLVLATGLRNSPLTETRGLFGAIAGFIEGGWQGMVDGWYGYHHSNEQGSGYAADKESTQKAIDGVTNKVNSIIDKMNTQFEAVGREFNNLERRIENLNKKMEDGFLDVWTYNAELLVLMENERTLDFHDSNVKNLYDKVRLQLRDNAKELGNGCFEFYHKCDNECMESVRNGTYDYPQYSEEARLKREEISGVKLESIGTYQ

SEQ ID NO: 9 - protein, 276 aa, Artificial
  The sequence is artificially synthesized.
IPLGVVHNNTLQVSDIDKLVCRDKLSSTSQLKSVGLNLEGNGVATDVPTATKRWGFRAGVPPKVVNYEAGEWAENCYNLDIKKADGSECLPEAPEGVRGFPRCRYVHKVSGTGPCPEGYAFHKEGAFFLYDRLASTIIYRSTTFSEGVVAFLILPETKKDFFQSPPLHEPANMTTDPSSYYHTVTLNYVADNFGTNMTNFLFQVDHLTYVQLEPRFTPQFLVQLNETIYTNGRRSNTTGTLIWKVNPTVDTGVGEWAFWENKKNFTKTLSSEELSV

SEQ ID NO: 10 - protein, 469 aa, Artificial
  The sequence is artificially synthesized.
MPLGVVTNSTLEVTEIDQLVCKDHLASTDQLKSVGLNLEGSGVSTDIPSATKRWGFRSGVPPKVVSYEAGEWAENCYNLEIKKPDGSECLPPPPDGVRGFPRCRYVHKAQGTGPCPGDYAFHKDGAFFLYDRLASTVIYRGVNFAEGVIAFLILAKPKETFLQSPPIREAVNYTENTSSYYATSYLEYEIENFGAQHSTTLFKIDNNTFVRLDRPHTPQFLFQLNDTIHLHQQLSNTTGRLIWTLDANINADIGEWAFWENKKNLSEQLRGEELSFEALSLNETEDDDAASSRITKGRISDRATRKYSDLVPKNSPGMVPLHIPEGETTLPSQNSTEGRRVGVNTQETITETAATIIGTNGNHMQISTIGIRPSSSQIPSSSPTTAPSPEAQTPTTHTSGPSVMATEEPTTPPGSSPGPTTEAPTLTTPENITTAVKTVLPQESTSNGLITSTVTGILGSLGLRKRSRR

SEQ ID NO: 11 - protein, 107 aa, Artificial
  The sequence is artificially synthesized.
VSYSLCTAAFTFTKIPAETLHGTVTVEVQYAGTDGPCKVPAQMAVDMQTLTPVGRLITANPVITESTENSKMMLELDPPFGDSYIVIGVGEKKITHHWHRSGSTIGK

SEQ ID NO: 12 - protein, 243 aa, Artificial
  The sequence is artificially synthesized.
NHKVTSTTTIIQDATSQIKNTTPTYLTQSPQLGISPSNPSEITSQITTILASTTPGVKSTLQSTTVGTKNTTTTQAQPSKPTTKQRQNKPPSKPNNDFHFEVFNFVPCSICSNNPTCWAICKRIPNKKPGKKTTTKPTEEPTFKTAKEDPKPQTTGSGEVPTTKPTGEPTINTTKTNITTTLLTSNTTRNPELTSQMETFHSTSSEGNPSPSQVSITSEYLSQPSSPPNTPRAHHHHHHHHHH

SEQ ID NO: 13 - protein, 168 aa, Artificial
  The sequence is artificially synthesized.
HHHHHHHHHHALEVLFQGPYEVRNVSGIYHVTNDCSNSSIVYEAADVIMHTPGCVPCVREGNSSRCWVALTPTLAARNASVPTTTIRRHVDLLVGTAAFCSAMYVGDLCGSIFLVSQLFTFSPRRHETVQDCNCSIYPGHVSGHRMAWDMMMNWSPTTALVVSQLLRI

SEQ ID NO: 14 - protein, 289 aa, Artificial
  The sequence is artificially synthesized.
ETHTTGRVAGHTTSGFTSLFSSGASQKIQLVNTNGSWHINRTALNCNDSLQTGFFAALFYAHKFNSSGCPERMASCRPIDWFAQGWGPITYTKPNSSDQRPYCWHYAPRPCGVVPASQVCGPVYCFTPSPVVVGTTDRSGVPTYSWGENETDMMLLNNTRPPQGNWFGCTWMNSTGFTKTCGGPPCNIGGVGNRTLICPTDCFRKHPEATYTKCGSGPWLTPRCLVDYPYRLWHYPCTLNFSIFKVRMYVGGVEHRLNAACNWTRGERCNLEDRDRSEAHHHHHHHHHH

SEQ ID NO: 15 - protein, 358 aa, Artificial
  The sequence is artificially synthesized.
DRICTGITSSNSPHVVKTATQGEVNVTGVIPLTTTPTKSHFANLKGTETRGKLCPKCLNCTDLDVALGRPKCTGKIPSARVSILHEVRPVTSGCFPIMHDRTKIRQLPNLLRGYEHIRLSTHNVINAENAPGGPYKIGTSGSCPNITNGNGFFATMAWAVPKNDKNKTATNPLTIEVPYICTEGEDQITVWGFHSDNETQMAKLYGDSKPQKFTSSANGVTTHYVSQIGGFPNQTEDGGLPQSGRIVVDYMVQKSGKTGTITYQRGILLPQKVWCASGRSKVIKGSLPLIGEADCLHEKYGGLNKSKPYYTGEHAKAIGNCPIWVKTPLKLANGTKYRPPAKLLKERAHHHHHHHHHH

SEQ ID NO: 16 - protein, 522 aa, Artificial
  The sequence is artificially synthesized.
DQICIGYHANNSTEQVDTIMEKNVTVTHAQDILEKTHNGKLCDLDGVKPLILRDCSVAGWLLGNPMCDEFINVPEWSYIVEKANPANDLCYPGNFNDYEELKHLLSRINHFEKIQIIPKSSWSDHEASSGVSSACPYQGTPSFFRNVVWLIKKNNTYPTIKRSYNNTNQEDLLILWGIHHSNDAAEQTKLYQNPTTYISVGTSTLNQRLVPKIATRSKVNGQSGRMDFFWTILKPNDAINFESNGNFIAPEYAYKIVKKGDSAIVKSEVEYGNCNTKCQTPIGAINSSMPFHNIHPLTIGECPKYVKSNKLVLATGLRNSPLTETRGLFGAIAGFIEGGWQGMVDGWYGYHHSNEQGSGYAADKESTQKAIDGVTNKVNSIIDKMNTQFEAVGREFNNLERRIENLNKKMEDGFLDVWTYNAELLVLMENERTLDFHDSNVKNLYDKVRLQLRDNAKELGNGCFEFYHKCDNECMESVRNGTYDYPQYSEEARLKREEISGVKLESIGTYQAHHHHHHHHHH

SEQ ID NO: 17 - protein, 514 aa, Artificial
  The sequence is artificially synthesized.
IPLGVVHNNTLQVSDIDKLVCRDKLSSTSQLKSVGLNLEGNGVATDVPTATKRWGFRAGVPPKVVNYEAGEWAENCYNLDIKKADGSECLPEAPEGVRGFPRCRYVHKVSGTGPCPEGYAFHKEGAFFLYDRLASTIIYRSTTFSEGVVAFLILPETKKDFFQSPPLHEPANMTTDPSSYYHTVTLNYVADNFGTNMTNFLFQVDHLTYVQLEPRFTPQFLVQLNETIYTNGRRSNTTGTLIWKVNPTVDTGVGEWAFWENKKNFTKTLSSEELSVADDDDKEPKSSDKTHTCPPCPAPELLGGPSVFLFPPKPKDTLMISRTPEVTCVVVDVSHEDPEVKFNWYVDGVEVHNAKTKPREEQYNSTYRVVSVLTVLHQDWLNGKEYKCKVSNKALPAPIEKTISKAKGQPREPQVYTLPPSRDELTKNQVSLTCLVKGFYPSDIAVEWESNGQPENNYKTTPPVLDSDGSFFLYSKLTVDKSRWQQGNVFSCSVMHEALHNHYTQKSLSLSPGK

SEQ ID NO: 18 - protein, 480 aa, Artificial
  The sequence is artificially synthesized.
MPLGVVTNSTLEVTEIDQLVCKDHLASTDQLKSVGLNLEGSGVSTDIPSATKRWGFRSGVPPKVVSYEAGEWAENCYNLEIKKPDGSECLPPPPDGVRGFPRCRYVHKAQGTGPCPGDYAFHKDGAFFLYDRLASTVIYRGVNFAEGVIAFLILAKPKETFLQSPPIREAVNYTENTSSYYATSYLEYEIENFGAQHSTTLFKIDNNTFVRLDRPHTPQFLFQLNDTIHLHQQLSNTTGRLIWTLDANINADIGEWAFWENKKNLSEQLRGEELSFEALSLNETEDDDAASSRITKGRISDRATRKYSDLVPKNSPGMVPLHIPEGETTLPSQNSTEGRRVGVNTQETITETAATIIGTNGNHMQISTIGIRPSSSQIPSSSPTTAPSPEAQTPTTHTSGPSVMATEEPTTPPGSSPGPTTEAPTLTTPENITTAVKTVLPQESTSNGLITSTVTGILGSLGLRKRSRRAHHHHHHHHHH

SEQ ID NO: 19 - protein, 345 aa, Artificial
  The sequence is artificially synthesized.
VSYSLCTAAFTFTKIPAETLHGTVTVEVQYAGTDGPCKVPAQMAVDMQTLTPVGRLITANPVITESTENSKMMLELDPPFGDSYIVIGVGEKKITHHWHRSGSTIGKADDDDKEPKSSDKTHTCPPCPAPELLGGPSVFLFPPKPKDTLMISRTPEVTCVVVDVSHEDPEVKFNWYVDGVEVHNAKTKPREEQYNSTYRVVSVLTVLHQDWLNGKEYKCKVSNKALPAPIEKTISKAKGQPREPQVYTLPPSRDELTKNQVSLTCLVKGFYPSDIAVEWESNGQPENNYKTTPPVLDSDGSFFLYSKLTVDKSRWQQGNVFSCSVMHEALHNHYTQKSLSLSPGK